European Patent Specification EP 3 479 852 B1, published May 31, 2023. Title: A porous biphasic scaffold for osteochondral composite tissue regeneration and a manufacturing method thereof. Applicant: Dankook University Cheonan Campus Industry Academic Cooperation Foundation. The sequence listing filed with the application follows.

SEQUENCE LISTING (8 sequences)

SEQ ID NO: 1 - DNA, 17 bp, Artificial
  Forward primer for the amplification of GAPDH gene
ctggaagatggtgatgg

SEQ ID NO: 2 - DNA, 19 bp, Artificial
  Reverse primer for the amplification of GAPDH gene
gatttggtcgtattgggcg

SEQ ID NO: 3 - DNA, 20 bp, Artificial
  Forward primer for the amplification of Aggrecan gene
tcgcaagtcccttccacatc

SEQ ID NO: 4 - DNA, 20 bp, Artificial
  Reverse primer for the amplification of Aggrecan gene
tcaaggcgtcctgaagtgtc

SEQ ID NO: 5 - DNA, 20 bp, Artificial
  Forward primer for the amplification of Collagen type II gene
gctggtgcacaaggtcctat

SEQ ID NO: 6 - DNA, 20 bp, Artificial
  Reverse primer for the amplification of Collagen type II gene
agggccagaagtaccctgat

SEQ ID NO: 7 - DNA, 20 bp, Artificial
  Forward primer for the amplification of Sox9 gene
ccagcaagaacaagccacac

SEQ ID NO: 8 - DNA, 20 bp, Artificial
  Reverse primer for the amplification of Sox9 gene
cttgcccagagtcttgctga